European Patent Specification EP 4 093 861 B1, published December 25, 2024. Title: Verfahren zum Nachweis von hormonell aktiven Verbindungen, Kit und deren Verwendung. Applicant: Universität Leipzig Technische Universität Dresden. The sequence listing filed with the application follows.

SEQUENCE LISTING (2 sequences)

SEQ ID NO: 1 - protein, 294 aa, Homo sapiens
MNSELDYYEKFEEVHGILMYKDFVKYWDNVEAFQARPDDLVIATYPKSGTTWVSEIVYMIYKEGDVEKCKEDVIFNRIPFLECRKENLMNGVKQLDEMNSPRIVKTHLPPELLPASFWEKDCKIIYLCRNAKDVAVSFYYFFLMVAGHPNPGSFPEFVEKFMQGQVPYGSWYKHVKSWWEKGKSPRVLFLFYEDLKEDIRKEVIKLIHFLERKPSEELVDRIIHHTSFQEMKNNPSTNYTTLPDEIMNQKLSPFMRKGITGDWKNHFTVALNEKFDKHYEQQMKESTLKFRTEI

SEQ ID NO: 2 - protein, 302 aa, Artificial Sequence
  fusion protein
MNSELDYYEKFEEVHGILMYKDFVKYWDNVEAFQARPDDLVIATYPKSGTTWVSEIVYMIYKEGDVEKCKEDVIFNRIPFLECRKENLMNGVKQLDEMNSPRIVKTHLPPELLPASFWEKDCKIIYLCRNAKDVAVSFYYFFLMVAGHPNPGSLPEFVEKFMQGQVPYGSWYKHVKSWWEKGKSPRVLFLFYEDLKEDIRKEVIKLIHFLERKPSEELVDRIIHHTSFQEMKNNPSTNYTTLPDEIMNQKLSPFMRKGITGDWKNHFTVALNEKFDKHYEQQMKESTLKFRTEILEHHHHHH